European Patent Application EP 4 407 043 A2, published July 31, 2024. Title: SYSTEM AND METHOD FOR SEQUENCING. Applicant: Life Technologies Corporation. The sequence listing filed with the application follows.

SEQUENCE LISTING (4 sequences)

SEQ ID NO: 1 - DNA, 23 bp, synthetic construct
  misc_feature 1..23: note = Synthetic DNA
  source 1..23: mol_type = other DNA
cctctctatgggcagtcggtgat

SEQ ID NO: 2 - DNA, 20 bp, synthetic construct
  misc_feature 1..20: note = Synthetic DNA
  source 1..20: mol_type = other DNA
ccatctcatccctgcgtgtc

SEQ ID NO: 3 - DNA, 20 bp, synthetic construct
  misc_feature 1..20: note = Synthetic DNA
  source 1..20: mol_type = other DNA
cctatcccctgtgtgccttg

SEQ ID NO: 4 - DNA, 34 bp, synthetic construct
  misc_feature 1..34: note = Synthetic DNA
  source 1..34: mol_type = other DNA
attcgagctgttcatctgtatcttgcgctaccaa